European Patent Specification EP 3 792 362 B1, published September 30, 2026. Title: method and kit for identifying state of colorectal cancer. Applicant: EXELLON MEDICAL TECHNOLOGY. The sequence listing filed with the application follows.

SEQUENCE LISTING (105 sequences)

SEQ ID NO: 1 - DNA, 1242 bp, Homo sapiens
gcacagccacagcctcctcgcctccccaaactcccagccaaggcgcgcggtggcgtcctcgcgccctcgctcgcgtccccgcccgccgcctgcgcaagccaggcatgaatgctgagacttgcgtctcttactgcgagtcgccggccgctgccatggacgcctactacagcccggtgtcgcagagtcgggagggctcgtcgccttttagggcatttcccggaggcgacaagttcggcacaactttcctgtcggccgccgccaaagcacagggattcggggacgccaagagccgggcccgttacggcgctgggcagcaggacctggcgacacccctggagagtggagctggggcgcggggctcctttaacaagttccagccccagccgtcgaccccgcagccccagccgccgccgcagccgcagccgcagcagcagcagccgcagccccagccgcccgcgcaaccgcatctttacttgcagcgaggcgcctgcaagacgcccccggacggcagcctcaaactccaggaaggcagcagcggccacagcgcggccttgcaggttccctgctacggtgagtgcacgtgcgggtcacctggtgctggggaccacggggtgcttggcttccgcatcccttgaaactggtggcttgcgggaggtatgagttggcgggctgggggcggggtggtgactctggtcggtaaacgggatcgatcgctgcgagggagccaagggatctgttctgtctccttcttgtccgccggcctaggcacggagcgtttcggctgttaaactcgacttggagtttgtttttcccggtcccttcggcatttccccaaaccgctcgctttgcgctgcccgctgggcgggatttgaagcggatgcttcttaccggcccagggcgtgcggcggcaaggagtctccgcgcagcgctctggcgctgggctgcggggctgcggggctgcggggctgcggggctgcggggctgcgaggctgcggggctgcggggctgcgggacagcaggactgcagaagcctcgctcctcgccggctgggaggctcctcgggcggcgccgccgcaggtgagagcgccgcaggtgcggagccaggcgggaagcccggagcgtggttggccgaaagctcacgggaaatccaggcgcactggcgcaacacagtgcggagccagagaccctagggtcccaggggacactgtggtctggcaagacccgagtcctgggaccctgagc

SEQ ID NO: 2 - DNA, 279 bp, Homo sapiens
cggacaaaaccataagtagttaccttcattgttccgtcggccacgagggaagctcgagctgagcggagggcagatcccaagggtcgtagcccctggccgtgtggaccgggtctgcggctgcagagcgcggtcccggctgcagcaagacctggggcagtgcccgaggcggcggcgagtacacgtggcgggctggattgcagaccggccctctcgcggcggagactcgcgacctagcggattgcatcagcaggaagacactaaggctgctcccccaggccg

SEQ ID NO: 3 - DNA, 427 bp, Homo sapiens
tcctagtccctcgcgcggccagtttggccgggtgttcccaaaaataaagcgaggagggaaggtacagacagatcttgaaaacacccgggccacacacgccgcgacctacagctctttctcagcgttggagtggagacggcgcccgcagcgccctgcgcgggtgaggtccgcgcagctgctggggaagagcccacctgtcaggctgcgctgggtcagcgcagcaagtggggctggccgctatctcgctgcacccggccgcgtcccgggctccgtgcgccctcgccccagctggtttggagttcaaccctcggctccgccgccggctccttgcgccttcggagtgtcccgcagcgacgccgggagccgacgcgccgcgcgggtacctagccatggctggggcgagcaggctgctctttctgtggctggg

SEQ ID NO: 4 - DNA, 470 bp, Homo sapiens
gcggcgaggggagggcccgggcgcggtgcgcgcgggggtggcggcggcgcgccgagcgggcccggcgcgggcgagcgggctgcagccggcggcggcgccagcaggtacggcccgcacccgccgccgccccggcggcctttgggggctgagccggagcccggcgcgattgcaaagttttcgtgcgcggcccctctggcccggagttgcggctgagacgcgcgccgcgcgagccgggggactcggcgacggggcggggacgggacgacgcaccctctccgtgtcccgctctgcgcccttctgcgcgccccgctccctgtaccggagcagcgatccgggaggcggccgagaggtgcgcgcggggccgagccggctgcggggcaggtcgagcagggaccgccagcgtgcgtcaccccaaagtttgcggggtggcagggcgcgcgctctggccacccgccgctctgggcggcagc

SEQ ID NO: 5 - DNA, 386 bp, Homo sapiens
ctcccccgggaacccgacgccgcgcggccacagggggcctggaggggcgggcagggcctcgcagcgcacccagcacagtccgcgcggcggagcgggtgagaagtcggcgggggcgcggatcgaccggggtgtcccccaggctccgcgtcgcggtccccgctcgccctcccgcccgcccaccgggcaccccagccgcgcagaaggcggaagccacgcgcgagggaccgcggtccgtccgggactagccccaggcccggcaccgccccgcgggccgagcgcccacacccgccaaacccacgcgggcacgcccccgcggcgcaccgcccccagcccggcctccgcccctgcagccgcgggcacgcggaggggctcctggctgcccgcac

SEQ ID NO: 6 - DNA, 552 bp, Homo sapiens
gaggcagagcccgggacctcgcgctctcgcctcaggctccggcccacgctcccgcccggccgccaggcgcgcaacggaaagcgcccccgccccgccccgctccgcccactgcgtgacgcgcacccggccgagccaatcagagctcgtggcgcgcgccccacacgccggccccctccgcccctcagcttaagaaagggcgcgcggacccggcaggccagagtgccgagcagcgcggtgggtgcggctgtgagacggcaggagacttctgccccgcggtgcacgcgaccctcgagacgacagcgcggctactgccagcagcgaaggcgcctcccgcggagcgccccgacggcgcccgctcgcccatgccgagctgagcgcggcagcggcggcgggatgctggcgctgctggccgccagcgtggcgctcgccgtggccgctggggcccaggacagcccggcgcccggtagccgcttcgtgtgcacggcactgcccccagaggcggtgcacgccggctgcccgctgcccgcgatgcccatgcagggcggcgcgcag

SEQ ID NO: 7 - DNA, 828 bp, Homo sapiens
acagacagaaaggcgcacagaggaatttaaagtgtgggctggggggcgaggcggtgggcgggaggcgagcgggcgcaggcggaacaccgttttccaagctaagccgccgcaaataaaaaggcgtaaagggagagaagttggtgctcaacgtgagccaggagcagcgtcccggctcctcccctgctcattttaaaagcacttcttgtattgtttttaaggtgagaaataggaaagaaaacgccggcttgtgcgctcgctgcctgcctctctggctgtctgcttttgcagggctgctgggagtttttaagctctgtgagaatcctgggagttggtgatgtcagactagttgggtcatttgaaggttagcagcccgggtagggttcaccgaaagttcactcgcatatattaggcaattcaatctttcattctgtgtgacagaagtagtaggaagtgagctgttcagaggcaggagggtctattctttgccaaaggggggaccagaattcccccatgcgagctgtttgaggactgggatgccgagaacgcgagcgatccgagcagggtttgtctgggcaccgtcggggtaggatccggaacgcattcggaaggctttttgcaagcatttacttggaaggagaacttgggatctttctgggaaccccccgccccggctggattggccgagcaagcctggaaaatggtaaatgatcatttggatcaattacaggcttttagctggcttgtctgtcataattcatgattcggggctgggaaaaagaccaacagcctacgtgccaaaaaaggggcagagtttgatggagttgggtg

SEQ ID NO: 8 - DNA, 828 bp, Homo sapiens
cggtgagcagagccggcgcagccacagcgcggagccgcggcgcccactggtcctcggagctgccaatcggcgtgtaatcctgtaggaatttctcccgggtttatctgggagtcacactgccgcctcctctccccagtcgcccaggggagcccggagaagcaggctcaggagggagggagccagaggaaaagaagaggaggagaaggaggaggacccggggagggaggcgcggcgcgggaggaggaggggcgcagccgcggagccagtggccccgcttggacgcgctgctctccagatacccccggagctccagccgcgcggatcgcgcgctcccgccgctctgcccctaaacttctgccgtagctccctttcaagccagcgaatttattccttaaaaccagaaactgaacctcggcacgggaaaggagtccgcggaggagcaaaaccacagcagagcaagaagagcttcagagagcagccttcccggagcaccaactccgtgtcgggagtgcagaaaccaacaagtgagagggcgccgcgttcccggggcgcagctgcgggcggcgggagcaggcgcaggaggaggaagcgagcgcccccgagccccgagcccgagtccccgagcctgagccgcaatcgctgcggtactctgctccggattcgtgtgcgcgggctgcgccgagcgctgggcaggaggcttcgttttgccctggttgcaagcagcggctgggagcagccggtccctggggaatatgcggcgcgcgtggatcctgctcaccttgggcttggtggcctgcgtgtcggcggagtcggtgagtgggccaggcg

SEQ ID NO: 9 - DNA, 572 bp, Homo sapiens
cggtgcgggtgcgggaacctgatccgcccgggaggcgggggcggggcgggggcgcagcgcgcggggaggggccggcgcccgccttcctcccccattcattcagctgagccagggggcctaggggctcctccggcggctagctctgcactgcaggagcgcgggcgcggcgccccagccagcgcgcagggcccgggccccgccgggggcgcttcctcgccgctgccctccgcgcgacccgctgcccaccagccatcatgtcggaccccgcggtcaacgcgcagctggatgggatcatttcggacttcgaaggtgggtgctgggctggctgctgcggccgcggacgtgctggagaggaccctgcgggtgggcctggcgcgggacgggggtgcgctgaggggagacgggagtgcgctgaggggagacgggacccctaatccaggcgccctcccgctgagagcgccgcgcgcccccggccccgtgcccgcgccgcctacgtgggggaccctgttaggggcacccgcgtagaccctgcgcgccctcacaggaccctgtgctcgttctgcgcactgccg

SEQ ID NO: 10 - DNA, 446 bp, Homo sapiens
gccactctcgctccgaggtccccgcgccagagacgcagccgcgctcccaccacccacacccaccgcgccctcgttcgcctcttctccgggagccagtccgcgccaccgccgccgcccaggccatcgccaccctccgcagccatgtccaccaggtccgtgtcctcgtcctcctaccgcaggatgttcggcggcccgggcaccgcgagccggccgagctccagccggagctacgtgactacgtccacccgcacctacagcctgggcagcgcgctgcgccccagcaccagccgcagcctctacgcctcgtccccgggcggcgtgtatgccacgcgctcctctgccgtgcgcctgcggagcagcgtgcccggggtgcggctcctgcaggactcggtggacttctcgctggccgacgccatcaacaccgagttcaagaacacccgcaccaa

SEQ ID NO: 11 - DNA, 18 bp, artificial sequence
tgcgtaagttaggtatga

SEQ ID NO: 12 - DNA, 18 bp, artificial sequence
ctacgacaccgaactata

SEQ ID NO: 13 - DNA, 31 bp, artificial sequence
tgtaagttaggtatgaatgttgagatttgtg

SEQ ID NO: 14 - DNA, 22 bp, artificial sequence
ccataacaacgaccgacgactc

SEQ ID NO: 15 - DNA, 20 bp, artificial sequence
gtaggattgtagaagtttcg

SEQ ID NO: 16 - DNA, 18 bp, artificial sequence
tacgccaatacacctaaa

SEQ ID NO: 17 - DNA, 25 bp, artificial sequence
gttttgttttttgttggttgggagg

SEQ ID NO: 18 - DNA, 20 bp, artificial sequence
caaccacgctccgaacttcc

SEQ ID NO: 19 - DNA, 24 bp, artificial sequence
tgttgatgtaattcgttaggtcgc

SEQ ID NO: 20 - DNA, 19 bp, artificial sequence
aatacccgaaacgacgacg

SEQ ID NO: 21 - DNA, 32 bp, artificial sequence
atttgttaggttgtgagtttttgttgtgagag

SEQ ID NO: 22 - DNA, 22 bp, artificial sequence
aaaccgaccctctcgcgacgaa

SEQ ID NO: 23 - DNA, 21 bp, artificial sequence
tttattgtttcgtcggttacg

SEQ ID NO: 24 - DNA, 20 bp, artificial sequence
cccaaatcttactacaaccg

SEQ ID NO: 25 - DNA, 31 bp, artificial sequence
tgttggttatgagggaagtttgagttgagtg

SEQ ID NO: 26 - DNA, 23 bp, artificial sequence
cgcgctctacaaccgcaaacccg

SEQ ID NO: 27 - DNA, 17 bp, artificial sequence
cgggttatatacgtcgc

SEQ ID NO: 28 - DNA, 16 bp, artificial sequence
ccaacaactacgcgaa

SEQ ID NO: 29 - DNA, 31 bp, artificial sequence
tacacaaacctcacccacacaaaacactaca

SEQ ID NO: 30 - DNA, 21 bp, artificial sequence
cgctacgaacgccgtctccac

SEQ ID NO: 31 - DNA, 18 bp, artificial sequence
ttgggttagcgtagtaag

SEQ ID NO: 32 - DNA, 18 bp, artificial sequence
ccaactaaaacgaaaacg

SEQ ID NO: 33 - DNA, 23 bp, artificial sequence
tgtagtaagtggggttggttgtt

SEQ ID NO: 34 - DNA, 23 bp, artificial sequence
cgaccgaatacaacgaaataacg

SEQ ID NO: 35 - DNA, 19 bp, artificial sequence
gtaggtacggttcgtattc

SEQ ID NO: 36 - DNA, 18 bp, artificial sequence
cgcacgaaaactttacaa

SEQ ID NO: 37 - DNA, 28 bp, artificial sequence
gtatttgtcgttgttttggtggtttttg

SEQ ID NO: 38 - DNA, 20 bp, artificial sequence
cgccgaactccgactcaacc

SEQ ID NO: 39 - DNA, 22 bp, artificial sequence
gacgggacgacgtatttttttc

SEQ ID NO: 40 - DNA, 16 bp, artificial sequence
cgcgcgcacctctcga

SEQ ID NO: 41 - DNA, 29 bp, artificial sequence
gggattgttagtgtgtgttattttaaagt

SEQ ID NO: 42 - DNA, 26 bp, artificial sequence
cgcctcccgaatcgctactccgatac

SEQ ID NO: 43 - DNA, 22 bp, artificial sequence
cgtagcgtatttagtatagttc

SEQ ID NO: 44 - DNA, 18 bp, artificial sequence
ccgataaacgaacgaaaa

SEQ ID NO: 45 - DNA, 27 bp, artificial sequence
atttagtatagtttgtgtggtggagtg

SEQ ID NO: 46 - DNA, 20 bp, artificial sequence
accgcgacgcgaaacctaaa

SEQ ID NO: 47 - DNA, 19 bp, artificial sequence
cgttcgggattagttttag

SEQ ID NO: 48 - DNA, 18 bp, artificial sequence
ccgcgtaaatttaacgaa

SEQ ID NO: 49 - DNA, 26 bp, artificial sequence
tgggattagttttaggtttggtattg

SEQ ID NO: 50 - DNA, 20 bp, artificial sequence
acccgcgaaacgataccgaa

SEQ ID NO: 51 - DNA, 20 bp, artificial sequence
cgtaacggaaagcgttttcg

SEQ ID NO: 52 - DNA, 26 bp, artificial sequence
tactcgacactctaacctaccgaatc

SEQ ID NO: 53 - DNA, 31 bp, artificial sequence
atggaaagtgtttttgttttgttttgttttg

SEQ ID NO: 54 - DNA, 25 bp, artificial sequence
accgaatacgcgtcacgcaataaac

SEQ ID NO: 55 - DNA, 20 bp, artificial sequence
attttcgagacgatagcgcg

SEQ ID NO: 56 - DNA, 23 bp, artificial sequence
tacacacgaaacgactaccgaac

SEQ ID NO: 57 - DNA, 34 bp, artificial sequence
ttgagatgatagtgtggttattgttagtagtgaa

SEQ ID NO: 58 - DNA, 21 bp, artificial sequence
tccgcgaaaaacgccttcgct

SEQ ID NO: 59 - DNA, 18 bp, artificial sequence
cggattcggtaggttaga

SEQ ID NO: 60 - DNA, 20 bp, artificial sequence
cgctatcgtctcgaaaatcg

SEQ ID NO: 61 - DNA, 26 bp, artificial sequence
aggttagagtgttgagtagtgtggtg

SEQ ID NO: 62 - DNA, 23 bp, artificial sequence
aatctcctaccgtctcacaaccg

SEQ ID NO: 63 - DNA, 25 bp, artificial sequence
gcgtatagaggaatttaaagtgtgg

SEQ ID NO: 64 - DNA, 27 bp, artificial sequence
acgcctttttatttacgacgacttaac

SEQ ID NO: 65 - DNA, 39 bp, artificial sequence
ttatttacaacaacttaacttaaaaaacaatattccacc

SEQ ID NO: 66 - DNA, 21 bp, artificial sequence
tattccgcctacgcccgctcg

SEQ ID NO: 67 - DNA, 27 bp, artificial sequence
gaatttttttatgcgagttgtttgagg

SEQ ID NO: 68 - DNA, 25 bp, artificial sequence
ttccgaatacgttccgaatcctacc

SEQ ID NO: 69 - DNA, 33 bp, artificial sequence
ttatgtgagttgtttgaggattgggatgttgag

SEQ ID NO: 70 - DNA, 26 bp, artificial sequence
aacaaaccctactcgaatcgctcgcg

SEQ ID NO: 71 - DNA, 21 bp, artificial sequence
tgggaatttttcgtttcggtt

SEQ ID NO: 72 - DNA, 29 bp, artificial sequence
acacgtaaactattaatctttttcccaac

SEQ ID NO: 73 - DNA, 34 bp, artificial sequence
cataaactattaatctttttcccaaccccaaatc

SEQ ID NO: 74 - DNA, 30 bp, artificial sequence
tcatttaccattttccaaacttactcgacc

SEQ ID NO: 75 - DNA, 19 bp, artificial sequence
cggcgtagttatagcgcgg

SEQ ID NO: 76 - DNA, 23 bp, artificial sequence
ccgaactcccctaaacgactaaa

SEQ ID NO: 77 - DNA, 33 bp, artificial sequence
agttatagtgtggagttgtggtgtttattggtt

SEQ ID NO: 78 - DNA, 30 bp, artificial sequence
tacaaaattacacgccgattaacaactccg

SEQ ID NO: 79 - DNA, 17 bp, artificial sequence
cgtaggaggaggaagcg

SEQ ID NO: 80 - DNA, 17 bp, artificial sequence
gcacacgaatccgaaac

SEQ ID NO: 81 - DNA, 29 bp, artificial sequence
ggaggaagtgagtgtttttgagttttgag

SEQ ID NO: 82 - DNA, 29 bp, artificial sequence
aataccgcaacgattacgactcaaactcg

SEQ ID NO: 83 - DNA, 22 bp, artificial sequence
cgagtttgagtcgtaatcgttg

SEQ ID NO: 84 - DNA, 21 bp, artificial sequence
caaccaaaacaaaacgaaacc

SEQ ID NO: 85 - DNA, 34 bp, artificial sequence
tgtaattgttgtggtattttgttttggatttgtg

SEQ ID NO: 86 - DNA, 21 bp, artificial sequence
aacgctcgacgcaacccgcgc

SEQ ID NO: 87 - DNA, 20 bp, artificial sequence
cgcgattcgttgtttattag

SEQ ID NO: 88 - DNA, 18 bp, artificial sequence
caccttcgaaatccgaaa

SEQ ID NO: 89 - DNA, 36 bp, artificial sequence
aaaatccaaaataatcccatccaactacacattaac

SEQ ID NO: 90 - DNA, 27 bp, artificial sequence
cgcgttaaccgcgaaatccgacataat

SEQ ID NO: 91 - DNA, 19 bp, artificial sequence
tagcgtattttcgtttcgc

SEQ ID NO: 92 - DNA, 25 bp, artificial sequence
cgaacttcgaaaataaatactaaac

SEQ ID NO: 93 - DNA, 32 bp, artificial sequence
tttgttttgtgttaggtttatttgtagggttt

SEQ ID NO: 94 - DNA, 22 bp, artificial sequence
aactactacgaccgcgaacgta

SEQ ID NO: 95 - DNA, 25 bp, artificial sequence
tcgtcgtcgtttaggttatcgttat

SEQ ID NO: 96 - DNA, 26 bp, artificial sequence
acgaataaacgtaatcacgtaactcc

SEQ ID NO: 97 - DNA, 40 bp, artificial sequence
gttgtttaggttattgttattttttgtagttatgtttatt

SEQ ID NO: 98 - DNA, 35 bp, artificial sequence
tacgataaaaaaacgaaaacacgaacctaataaac

SEQ ID NO: 99 - DNA, 25 bp, artificial sequence
gtcgtagtttttacgtttcgttttt

SEQ ID NO: 100 - DNA, 31 bp, artificial sequence
tacgaatattcttaaactcgatattaataac

SEQ ID NO: 101 - DNA, 30 bp, artificial sequence
ttatgttttgtttttgggtggtgtgtatgt

SEQ ID NO: 102 - DNA, 21 bp, artificial sequence
aacacgctactccgcaaacgc

SEQ ID NO: 103 - DNA, 23 bp, artificial sequence
gtgatggaggaggtttagtaagt

SEQ ID NO: 104 - DNA, 23 bp, artificial sequence
ccaataaaacctactcctccctt

SEQ ID NO: 105 - DNA, 30 bp, artificial sequence
accaccacccaacacacaataacaaacaca